European Patent Application EP 4 803 086 A1, published September 9, 2026. Title: Adiponectin enhancer, oral composition for enhancement of adiponectin and use of plasmalogen. Applicant: INSTITUTE OF RHEOLOGICAL FUNCTION OF FOOD CO., LTD. Application WO. The sequence listing filed with the application follows.

SEQUENCE LISTING (4 sequences)

SEQ ID NO: 1 - DNA, 20 bp, synthetic construct
  source 1..20: mol_type = other DNA
ctgtccccatgagtaccaga

SEQ ID NO: 2 - DNA, 20 bp, synthetic construct
  source 1..20: mol_type = other DNA
taacgtcatcttcggcatga

SEQ ID NO: 3 - DNA, 20 bp, synthetic construct
  source 1..20: mol_type = other DNA
accacagtccatgccatcac

SEQ ID NO: 4 - DNA, 22 bp, synthetic construct
  source 1..22: mol_type = other DNA
tccaccaccccctgttgctgta